European Patent Application EP 4 717 088 A1, published April 1, 2026. Title: METHOD FOR IMPROVING PLANT CULTIVATION UNDER ABIOTIC STRESS CONDITIONS. Applicant: Timac Agro España, S.A. Application EP 24782600.1, filed July 16, 2024. The sequence listing filed with the application follows.

SEQUENCE LISTING (2 sequences)

SEQ ID NO: 1 - DNA, 4594 bp, Solanum lycopersicum
  source 1..4594: mol_type = genomic DNA
gcagtttcttcaggcactgtatttagaatcaaccagcacccaagttctccatacatgaaaactccaagattttacaacttcacaaagaaaaaagtgagtaaataagataccccatttgattttcttgaaaaaatttgtgtttttttcatgtaaagttttgatcttttgtggaattctggtaaaattttcttattcccacatattttggaatggatttgtttgagtttttttgtaaagttgtgatctttttaaaacttttatgatatctggtactgatatattcttgttttttcagtttctttgtatatggtttatgtaaagttataatcttttgatataatcatatctatttatctagagctcttgaaatgtccctttttcagtttcttgtaaaagtttatttaaagttgtgatcttttgtacgatctgcgttttaatttgtttgtctaattctgagttgatgtgaagtttaagaaggtaaagaagaatttaaattttgaatcttgtgttgttaaataaaagatacgtagattgtaccaaaatgttctttaatctctaacgtctttacatgaaaagttatagttagatagtcgtaaaaaaaaaaaggaaagtgacattttttttaaacagactaaaagaaaaagtaagacgaacagtattagcatcttgaagtgttttttgtctcatttcttgtaaaatcttttgtaatgttatgatcttttgtaacctttttggtataatcatttggtatctggaacgcactagcctcgactaaaattgatgtttttgtttcagtttcttgtaaaagcttctgtgaatggctcagatgaaatcaatgggaagatagtaagaaaggaagaaaaagatagtttgcagattgatttttcaggtgaaaagccacctacaccatttttggatacaatcaattatcctaaacatatgaagaatctatcaaaaatggtaaattccttatcaaacaattaaatattaagccttttatcggattatttgatcgatatgcatttttttcgaataaaaaacaggatcttgaacagttagctgcagaactaagagcagagattgtgtattcagtggcaaaaaccggaggtcatttgagttcaagtttaggtgttgtggatttaactgtggctttgcatcatgtttttgatactcctgaggataaaattatatgggatgttggtcatcaggtgaataaatctttattcttctttatttccttgaagaatagatagtttaatatggagtttatggtcaaaacacacctgaagtatcctggtttttgagctccatacctgaacgatcaggtattcgagtttcctacctggactatcaccatatatttatcgaaacacatccaactgtcaattattcacttttcttatccgaaatatcaccactgttcaggcaagaaaactgacaattgatagttaatgtttcgataaacgtttagtgatagttcaggtagaaaactcgcacacctatagttcaagtgtgaaacttgaaaaaaacggaatagttttgatgtgtttttgaccattcactcttttatatatatagtggaaattgaagtgaacaaaaaaaaattgcaggcatatgcacacaaaatcttgacaggaagaaggtctaaaatgcatacaatgagaaagacttcagggctagcaccttttcctaaaagggatgaaagtgttcatgatgcatttggtgcagggcatagttcaacaagcatctccgctggtcttggtaataaattcagttcatgacttcttcgctgctgtatttgctttacatactcgagctgagggtctattggaaacaacctctctaccttcacaaggtaggggtaaggctgcgtacacattaccctccctagacctcacttatgggattatactgggaatgttgttgttgttgttgtataacggtacaagttcaactgtcaaagtattgtccgctctggcctgacttttggggtctcgcggttctgtcagccgttttttgcattaaaggtgatgtgacagttgagttcttgatttgccttgtatggttcctaactttcccctcgcgttccaatgtgagattttctcttcacattgaaccccttttgagttcagagatccgttgattgttacatacttccattaggagaaaaagttgatgaatcccaagtacatgatttggagtttgtctaagttaaatgatgttttgcaggcatggcggttgctcgagatcttttagggaacaacaaccatgtcatatctgtaattggagacggagccatgactgcaggacaagcatacgaggccatgaataatgcaggattccttgactcgaatctgatagtcatattgaatgataataaacaagtttctttaccgaccgcaactttagatggccctgcaactccagtaggagccctcagtagtgccttaagcaaactccaagctagtcttaagtttaggcaactccgcgaagctgcaaaggtaaatctagttcatttttttcgcatacttatagttgtattcgaggattgaaatgaagtaaaggtgttaaaagtactttattcaatgtgttttgtagactataacaaagcaaattggacctcaagcacatgaagttgcagctaaagttgatgaatatgcaaggggaatgcttagtgcatctggttccacactttttgaggagctaggattatattacatcggtccagtagacggacacaatatcgaagacttgatcactattttagagaaggtaaaagcattgccagcaccaggaccagttctaattcacattgtaacagagaaagggaaaggttatcttcctgcagaagcagcagacgataaaatgcatggtaaggcaattggaaataagaagattacttgtttaaaattttgaaaaactgagatttttcgtttgtgatgttcaggggtggcacagtttgatccgaaaacaggaaagcaatttaaggccaagtcgcctacgttgacatatactcagtactttgctgaatcactgattaaagaagccgaaaatgataacaagattgtagctatccatgctgcaatgggtggtggaaccggcctcaattatttccaaaaacaatttccagaacgttgttttgacgttggcattgctgagcaacatgcagttacttttgcagcaggcttagctacagaaggtctaaaaccattttgtgctatctactcctcgttcttacaacgaggctacgatcaggtaactaacaacatacaaatagtaacatttgaagcactctacaatataagtcttgcattttcggattgctgtactaacattgcatatttgtaaaaaaaggtggtgcacgatgtggatcttcagaagttacctgtccggtttgcaatggaccgagctggtttggtaggtgcagacggtccaacgcattgtggagcattcgatgtgacatacatggcttgtttgccaaatatggtagtcatggctccatcggacgaagcagagctaatgcacatggttgcaacagcagcagctattgatgataggcctagttgtttccgatttcctagaggaaatggaattggtgcaattcttcctctaaacaataaaggcataccaattgaggtaacttaaaagtctgtttgaacacttgatgttttatcagctaatccaaacggactctaaattacattggcctttttgtctatgttgtaacatcaacaggtcggtaaaggaagaatactgagagaaggtgaaagagttgccattttgggatatggttcgataatacaacaatgtttgggagctgcagacatcctaaactcccatgacataagagtaacagtagctgatgctaggttctgcaaaccattggatgctgatcttattaggagtttagccaaagaacatgaaatcttgatcactgtcgaagaaggatcaatcggaggatttggctcacacgtgtctcatttcttaagcctaaacagcattttggacggaccccttaaggtaaaaatcactaacaaatctgtagttggaacgacaaaagtcatttttcaagaaaatattttttaagctatgttgtgtggattctctagccgagcgtctttcagaaacctccacgatgtaggggtaacattggatatgctattttatgtggactcatcaaaaatgttgttgcctcgtgccagatcctccaaaaatgctctacttccggaggatccaacaagcacttaacaatgttaaacatgacattctccttttaaacagatcaaaaaggaaagtaattaagacacaaaataaaatcgtaagaaacattttctatgtctatggaaaatgacttccgtcatatcaaacatgttcaaaaattataaattattgatttatttccattttttttcaataattttaatttttaaaccttgactttttgcagttgaggtcaatgttacttccagatagatacattgatcatggttcaccagttgatcaaattgaagcagctggtttatcatcaagacatatttcttctacagttctaacattattgggaaggccaaaagaagctatggtagtaaactaa

SEQ ID NO: 2 - DNA, 3150 bp, Solanum lycopersicum
  source 1..3150: mol_type = genomic DNA
tgggcgtgtccccaaattgtagcgcgccaaccgcttttcactctataaatacatttcttctactttcgcttctccacacaaaccatcactgcttaatacacatttgactttctctctctctcatttctctttttttttcttttcaaaaagccggtgttcctgccggaaaatcaactaaatttacaatggacgttcgccggcgaccagttaagcctttatgcacatcaaaagatgcttccgccggcgaacctctgaaacaacaacaagtttcttctcctaaagcatctgacgcgcttccactcccattgtacctaaccaatgggttgtttttcaccatgtttttctctgttatgtattttcttctcgtaaggtggcgtgagaagatccgtaattctattcctcttcatgtggttaccctttctgaattgttagctatggtgtcattgattgcttccgttatatatctattgggtttctttgggattgggtttgttcagtcgtttgtgtccaggtcgaatagtgattcatgggatattgaggatgagaatgctgagcagctaattatcgaggaagatagccgccggggaccatgtgctgctgcaactactcttggctgcgttgtgcctccaccacctgttcgaaaaattgccccaatggttccacagcaacctgccaaggcagctttgtcccaaacggagaagcctgcgccaataattatgccagcattatcggaagatgacgaggagataatacaatctgttgttcagggtaaaacaccatcatattctttggaatcaaagcttggtgattgtatgagagctgcttcgattcgaaaagaggcgttacagaggatcacagggaagtcattggaagggctcccattggaaggatttgactatgagtctattcttggacaatgctgtgagatgcctgtaggatatgtgcaaataccggttggtattgcagggcctttgttgcttgatgggagagagtactcagtgccaatggcaactacagaagggtgtttagttgctagcaccaacaggggttgcaaggctatctttgtctctggtggcgccaacagcattttgctcagagatggcatgacaagagctccggttgtccggttcaccaccgccaaaagagccgcagagttgaaattcttcgttgaggatccccttaactttgagattctttctcttatgttcaacaagtgagttttcttctcatgattacgtatattcttaattgtttcttctacgagtactagctattcgtaattggtgagctttttgttaaaagattggaggatgcttaccattttagcaatccgttgttggtgagagttagtatgaaacaattaagacaaaacatttaagttttgcttctctcttaattctatatcttgattcaatattttctgttacaaattctttattcaccagcaaagagaaaagaaatgatttgtcatatctagtatcctaattgaaagcttatgttaaaagttacatgtcatgtgcatttttattcaatattatgttttcaaaatttaaaatttgtttctgtaatggaaatttttgcagatcaagcagatttgctcgattacagggcattcaatgtgctatagctggtaaaaatctgtatatgagattcagttgtagcactggtgatgcaatgggaatgaacatggtatccaaaggtgtccagaacgttctggattaccttcagagtgaatatccagacatggacgtcattggcatatctggtattattccatcgacctgtttatgcatagttttttcccgcaacttgatgcacgagatgtttatttaattgagaatcatgtgaaatattgacagggaacttttgttcggataagaagccagcagcagttaactggattgaaggtagaggaaaatcagtagtttgcgaggcaataatcaaggaggatgtagtgaagaaagtgttgaaaactgaggttgctgctcttgtggagctgaacatgcttaaaaaccttactgggtcagccatggctggtgccctcggtggcttcaatgctcatgccagcaacatcgtctctgctgtatatttggccactggccaagaccctgctcaaaatgttgagagctctcactgcattactatgatggaggctgtaaatgatggcaaagacctccatatttcagtaactatgccttctattgaggtatacaaccaacatgctcctattattatgctctccatttcatattagttgtgcattttactaaaaataattgtctcaaattagttacattttaccgttacaatatcattttcgtaaatttttaacagaatttcttcatggatgtctagaggtgaaagtgaacaactaatatgaaattctaactagaggtgaaagtgaacaactgatatgagacgcttaccagtgcatgtaggctttgatctcatttaattgtagtagaataagtccagatgaaatattgacatgtagcatccttgacatttaatgagtgagaacctgtcattgtagcaggcaggttaggtgtgtcctgagtcagtccataattaagtggcatgcgaaggaagagacaaagttgcacatgttttatacacattagctaatttgtcctgtgaatttcaggttggtaccgtaggtggtggaactcaacttgcatcacagtcagcttgcttgaacttactaggagttaaaggtgcaaatagagatgcaccaggttcaaatgcaagactgttggccacaatagtagctggttctgttctagctggtgagctatctctcatgtcagctatctctgctggccaactagttaaaagtcacatgaaatataatagatctatcaaagatatttcccaagtaatcaattcctcttgaggattaattagccccccccccccccccaataaaaagaaagaataggaataaaattttcagaattagggagatctagctgcagcagaagaagtactttgaaccaaaattataatataaaagtaatgtattaaagatcttctttgttcatgaattaataatgtggggaatattcaagaacaagttggaatgtgttgtatgtattttttctatgaagccatgtgagggtgtagggtctctttgtttctgcaaatattata